European Patent Application EP 4 624 580 A1, published October 1, 2025. Title: MICROORGANISMS FOR PRODUCING PURINE NUCLEOTIDES AND PROCESS FOR PRODUCING PURINE NUCLEOTIDES USING THE SAME. Applicant: CJ CheilJedang Corporation. The sequence listing filed with the application follows.

SEQUENCE LISTING (56 sequences)

SEQ ID NO: 1 - DNA, 38 bp, synthetic construct
  source 1..38: mol_type = other DNA
aattcgagctcggtacccgttgccgtatcagacatgct

SEQ ID NO: 2 - DNA, 35 bp, synthetic construct
  source 1..35: mol_type = other DNA
tcataggtgccgaacttgatttatctcgaccaaac

SEQ ID NO: 3 - DNA, 35 bp, synthetic construct
  source 1..35: mol_type = other DNA
gtcgagataaatcaagttcggcacctatgagaata

SEQ ID NO: 4 - DNA, 38 bp, synthetic construct
  source 1..38: mol_type = other DNA
cgactctagaggatccccctcgggttccatgttgtctt

SEQ ID NO: 5 - DNA, 20 bp, synthetic construct
  source 1..20: mol_type = other DNA
cttgtgcgccgaagcccgtt

SEQ ID NO: 6 - DNA, 20 bp, synthetic construct
  source 1..20: mol_type = other DNA
gctttcatgagcttgccggg

SEQ ID NO: 7 - DNA, 38 bp, synthetic construct
  source 1..38: mol_type = other DNA
aattcgagctcggtacccaatccatcctgcgtcagaag

SEQ ID NO: 8 - DNA, 35 bp, synthetic construct
  source 1..35: mol_type = other DNA
cgctgggatgtttctggttgctcctttttattatt

SEQ ID NO: 9 - DNA, 35 bp, synthetic construct
  source 1..35: mol_type = other DNA
taaaaaggagcaaccagaaacatcccagcgctact

SEQ ID NO: 10 - DNA, 35 bp, synthetic construct
  source 1..35: mol_type = other DNA
gatataagactccaagagtgtttcctttcgttggg

SEQ ID NO: 11 - DNA, 35 bp, synthetic construct
  source 1..35: mol_type = other DNA
cgaaaggaaacactcttggagtcttatatcggtag

SEQ ID NO: 12 - DNA, 38 bp, synthetic construct
  source 1..38: mol_type = other DNA
cgactctagaggatcccccatcgctttatcagaaggac

SEQ ID NO: 13 - DNA, 20 bp, synthetic construct
  source 1..20: mol_type = other DNA
cgaatacctccagaccaccg

SEQ ID NO: 14 - DNA, 20 bp, synthetic construct
  source 1..20: mol_type = other DNA
tgggcacaacggtgacagcg

SEQ ID NO: 15 - DNA, 38 bp, synthetic construct
  source 1..38: mol_type = other DNA
aattcgagctcggtacccaggcacagccgacattacgg

SEQ ID NO: 16 - DNA, 35 bp, synthetic construct
  source 1..35: mol_type = other DNA
gtagcacatctgacgaatgtccaagtctaaggaaa

SEQ ID NO: 17 - DNA, 35 bp, synthetic construct
  source 1..35: mol_type = other DNA
ttagacttggacattcgtcagatgtgctacttgcc

SEQ ID NO: 18 - DNA, 35 bp, synthetic construct
  source 1..35: mol_type = other DNA
tgcgccattagcgtgttacttctcgcggctataga

SEQ ID NO: 19 - DNA, 35 bp, synthetic construct
  source 1..35: mol_type = other DNA
agccgcgagaagtaacacgctaatggcgcattgaa

SEQ ID NO: 20 - DNA, 35 bp, synthetic construct
  source 1..35: mol_type = other DNA
tgaattatccgcgtcttagatgccgttttctgccg

SEQ ID NO: 21 - DNA, 35 bp, synthetic construct
  source 1..35: mol_type = other DNA
gaaaacggcatctaagacgcggataattcagctgt

SEQ ID NO: 22 - DNA, 38 bp, synthetic construct
  source 1..38: mol_type = other DNA
cgactctagaggatccccgatgaagcgaacacttaaat

SEQ ID NO: 23 - DNA, 20 bp, synthetic construct
  source 1..20: mol_type = other DNA
ccagtacattgtcatgggat

SEQ ID NO: 24 - DNA, 20 bp, synthetic construct
  source 1..20: mol_type = other DNA
gattggcatatcgcaccgag

SEQ ID NO: 25 - DNA, 38 bp, synthetic construct
  source 1..38: mol_type = other DNA
aattcgagctcggtaccccatttcgtgaccattagcgt

SEQ ID NO: 26 - DNA, 35 bp, synthetic construct
  source 1..35: mol_type = other DNA
attagcctgaaggaagatcatgccaatagcgccag

SEQ ID NO: 27 - DNA, 35 bp, synthetic construct
  source 1..35: mol_type = other DNA
gctattggcatgatcttccttcaggctaatctttt

SEQ ID NO: 28 - DNA, 35 bp, synthetic construct
  source 1..35: mol_type = other DNA
attctgggtagtcatcatatgtgtttcctttcgtt

SEQ ID NO: 29 - DNA, 35 bp, synthetic construct
  source 1..35: mol_type = other DNA
aaggaaacacatatgatgactacccagaattcttc

SEQ ID NO: 30 - DNA, 35 bp, synthetic construct
  source 1..35: mol_type = other DNA
ctttgtacttggtgaccaagagtcaggatgccgaa

SEQ ID NO: 31 - DNA, 35 bp, synthetic construct
  source 1..35: mol_type = other DNA
catcctgactcttggtcaccaagtacaaagagact

SEQ ID NO: 32 - DNA, 38 bp, synthetic construct
  source 1..38: mol_type = other DNA
cgactctagaggatccccggttaccgcgcattaggact

SEQ ID NO: 33 - DNA, 20 bp, synthetic construct
  source 1..20: mol_type = other DNA
taatcccccagctcaccggc

SEQ ID NO: 34 - DNA, 20 bp, synthetic construct
  source 1..20: mol_type = other DNA
tttggatgccgaggtcgtag

SEQ ID NO: 35 - DNA, 40 bp, synthetic construct
  source 1..40: mol_type = other DNA
acccggggatcctctagagacatgctcagcacctttcttc

SEQ ID NO: 36 - DNA, 20 bp, synthetic construct
  source 1..20: mol_type = other DNA
agccttaaggctaccggatc

SEQ ID NO: 37 - DNA, 40 bp, synthetic construct
  source 1..40: mol_type = other DNA
tccggtagccttaaggctatgccggatttcgacgagtatc

SEQ ID NO: 38 - DNA, 38 bp, synthetic construct
  source 1..38: mol_type = other DNA
aagcttgcatgcctgcagcgccttcaaggacgcctaag

SEQ ID NO: 39 - protein, 361 aa, Corynebacterium stationis
MTATTNHLTENSHAHGYDHYQRMAFFTDTSVCIGCKACEVACKEWNRNPVEGYNLTGNSYDNTGALGANTWRHVAFIEQDNERITKAREEGAKLVSLGMPTIGTSPVDAAPNPASADTTPPDTDTFRWLMSSDVCKHCTNAGCLDVCPTGALFRTEFGTVVVQDDVCNGCGTCVAGCPFGVIERREDGGVSLKANHVEAQEVPEHAGINVFKKLKQLRPQGPDHVPGETMPIKNIGVAQKCTMCYDRLKVGEQPACSKTCPTESIQFGTYENMLAAAQARVAELHRQGQTEARLYGANNEDGVGGTGSIFLLLDSPEVYGLPPDPRVPTADLPAMAKTFAKAVGAMGVAVAASFLVDRGGT

SEQ ID NO: 40 - DNA, 1086 bp, Corynebacterium stationis
  source 1..1086: mol_type = genomic DNA
atgacggctacgaccaatcacctaacagaaaattcgcacgcgcacggctacgaccattaccagcgcatggcctttttcaccgatacttcggtgtgcattggctgtaaggcttgcgaggtggcctgtaaggagtggaaccgcaacccggttgagggctataacctgacgggtaattcctacgacaacaccggcgcgctgggcgcgaatacctggcgacacgtagcatttattgagcaagacaacgagcgcatcaccaaagcgcgtgaagaaggtgccaagctggtctcgctgggcatgccgacgattggcacttcgcctgtcgatgcagccccgaatcctgcctccgccgataccacgccgccggatactgatactttccgttggctgatgtcttctgatgtctgcaagcactgcaccaacgctggctgcctggatgtgtgcccaaccggtgctttatttcgcaccgaatttggcaccgtcgtggtccaagatgatgtctgcaatggctgcggcacctgcgttgccgggtgcccgttcggtgttattgagcgccgtgaagacggcggtgtttcgctaaaagccaaccacgtcgaagcccaagaagtccctgaacacgcgggcattaacgtgtttaagaagctcaaacagctgcgcccgcaaggaccggatcacgtcccgggtgagaccatgccgattaaaaatattggcgtggctcaaaagtgcaccatgtgctacgaccgcctgaaagtcggcgagcagccagcgtgttccaagacatgcccgacggagtccatccagttcggcacctatgagaatatgctggccgctgcgcaagcgcgcgtggctgagctacaccgtcaaggccagactgaggcacgactgtacggcgcaaataacgaagacggcgtcggcggaacgggctccatcttcttgctgctggattccccggaagtctacggtcttccaccagatccgcgtgtgccgactgcagatttgcccgcaatggcgaagactttcgccaaggccgttggcgccatgggcgttgccgtggcagcgtcctttttagttgatagaggagggacctag

SEQ ID NO: 41 - protein, 923 aa, Corynebacterium stationis
LGTSFGRGGATQPLQDMANADCILIQGSNMAECHPVGFQWVVEAKKRGARVIHVDPRYTRTSAFANRHVAIRGGTDVVLLGALIKYMIDNDLYFHDYVVNYTNASSIISPDFRDTEDLDGLFSGYNPETGKYITDSWQYVQKPEGAWWNIERDETLQDPNTVFQILKRHYSRYTPEIVEETCGISQEDFHYLAESIAQNSNPERTTVFAYALGFTQQTLGVQFIRAAAILQLLMGNVGRPGSGIMALRGHASIQGSTDIPTLFNNLPGYLPMPHADHGDWKGFLDAIAKEDQKGFWGLRENYAVSLMKSYWGENATKDNDWGWNYMPRINGAHSTYETLMGMLDGIVEGYIVFGQNPAVAQSNGGMQRRGLASLKWLVVRDFQEIETASFWYDSPEIKTGELKTEDIGTEVFLLPAATHVEKAGTFTQTQRMLQWRFQATNPPGDAKSDLWFFYQMGKRIREKLAGSTDPMDAPLLAIDWNYEETEHGEPDPEDVLREINGYYLDGPKKGQLLPGFTEMKPDGTTSGGCWIYSGVFKDNINQSARKVSGASQNEVALEWGWVWPSNRRMLYNRASAAPDGTPWSERKKYIWWDAEAGRWTGDDVPDFPVNLDPSYRAPVDATGPAALDGTDAFIMQADGRGWLFVPKGLSDGPLPTHYEPHESPARNILYSQQQSPTRLTIKRPDNLSKPMAGEPGSEVYPVVFSTYRLTEMYTSGAMSRRLPYLAELQPDLFVEVDPVLAQKRGLENGGWATIISPRGVIEARVLVTERMESMTINGKDFHQIGLPFHYGQSSSSPVTGDGANDLLGLTLEPNVFIQNSKVGACEIKAGRRPRGKARLEMLKEYQRRAGLTLDTGNELIDPDAQQLEATSTIDLFIPNGVDKETVETSTSEPGAADGSAHHGSAMGEVPNSEPKDTEGGEKQ

SEQ ID NO: 42 - DNA, 2772 bp, Corynebacterium stationis
  source 1..2772: mol_type = genomic DNA
ttgggaacctcgtttggccgcggtggcgcaactcagccactgcaggatatggcaaatgccgactgcatcctgattcagggctcgaatatggccgagtgccatcctgtgggtttccagtgggtagtcgaagctaaaaagcgcggggcgcgcgtaattcacgtggatcctcgctatacccgtacctcggcgtttgcgaaccggcacgtagcgatccgtggcggcaccgatgtggtgcttcttggcgcacttatcaagtacatgatcgacaatgatctgtattttcacgactatgtggtcaattacacgaacgcgtcgtcgatcatttctcccgacttccgggacacggaagacctagacggcctcttttctggctacaacccagaaaccggtaagtacatcacggactcgtggcagtacgtgcaaaagcccgaaggtgcgtggtggaatatcgagcgtgatgagactttgcaggacccgaatacggtcttccagattctcaagcgccactattcccgctataccccggaaatcgtggaagagacctgcggtatctcccaggaggacttccattatctagcggagtcgattgcacagaactccaatccagagcgcactacagtctttgcctatgctttgggctttacgcagcaaaccttaggcgtgcagttcattcgtgccgcggccatcttgcaactgctgatgggcaacgtgggccgcccgggctcaggcatcatggcgctgcgtggacacgcttccattcagggctcgacagatatcccgacgctgtttaataacttgccgggttacttgccgatgcctcatgccgaccatggcgactggaaaggattcttggacgcgattgccaaggaagaccagaagggtttctggggtctgcgtgaaaactatgccgtgagcttgatgaagtcctattggggcgagaatgccaccaaggacaatgactggggctggaactacatgccgcgcatcaacggtgcgcactccacctatgaaaccttgatgggcatgctcgacggcatcgtcgaaggctatatcgtcttcggacaaaacccagcggtcgctcaatccaacggcggcatgcaacgccgcggattggcgtctttgaagtggttggttgttcgtgacttccaggaaattgagacagcgtcattctggtacgactcaccagagatcaagactggtgaactcaagaccgaagatattggcaccgaggtcttccttcttcctgcagcaacgcacgtagaaaaggccggtacctttacccaaacccagcgcatgctgcagtggcgtttccaggccacaaatccaccaggcgatgccaagagcgatctgtggttcttctaccagatgggcaagcgcattcgcgaaaagcttgctggttctactgatccgatggacgcgccattgttggccatcgactggaactacgaggaaaccgaacacggcgagccagatcccgaagacgtgctgcgcgaaatcaacggctactatctggatggcccgaagaaggggcagctgctgcctggctttacagagatgaagcctgatggcacgacgtctggtggctgctggatctactccggcgtgttcaaggacaacatcaaccagtccgcgcgcaaagtttcaggcgcttcgcaaaatgaggttgcgctggaatggggctgggtatggccatcgaatcgccgcatgctgtacaaccgtgcgtcagctgcgccagacggcacgccatggtcggagcgcaagaagtacatttggtgggacgctgaggccggccgctggacgggcgacgacgtaccggacttcccagtcaacttggatccgtcataccgcgcgcctgtcgatgccacaggtcctgcagcccttgacggcaccgatgcgtttatcatgcaggcagatggtcgtggttggttgttcgtacccaaaggactttccgatggacccctgccaacccactatgaaccgcacgagtcgccggcacgcaatattttgtacagccagcagcagtcgccgacacgcttgaccatcaagcgtccggataacttgtcgaagcccatggctggtgagcccggctcagaggtctaccccgtggttttctccacgtaccgtttgacggagatgtacacctcgggtgcgatgagccgccgactgccttatttggcagagttgcagccagatttgttcgttgaggtcgatccggttctagcacaaaagcgcggcttggaaaacggtggctgggcaaccatcatttcgccgcgtggcgtgattgaggctcgcgtgctggtgaccgaacgcatggaatctatgaccatcaatggcaaggacttccaccagattggtctgcctttccactacggtcagtccagctcctcgccagttactggtgacggtgccaatgaccttctgggtctaactttggagccgaatgtgttcattcaaaactccaaggttggtgcatgtgaaattaaggccggccgacgcccacgcggcaaggcgcggttagagatgctcaaggaataccagcgccgtgccggattgacgttggacaccggtaacgagctcatcgatcccgatgcacagcagctcgaagctacctccacgatcgacttatttattccgaatggcgtagacaaagagacggtggagacatcgacaagcgagcctggcgccgcagatggttctgcgcatcatggctcagcgatgggggaagtcccaaattctgaaccaaaagatacggagggaggcgaaaagcaatga

SEQ ID NO: 43 - protein, 188 aa, Corynebacterium stationis
MSKLSPLNWPVVRQVKRGDLFGRDKSTQSAKSENLHGRTVEADKVVQSVCPYCAVGCSQRVYVKDDRVVHIEGDSDSPISRGRLCPKGAASEQLVNSATRLTKIKYRAPHATEWQDLDLETAMDMIADRFIASRRNQWQDFDEKGRVLNRTMGVAGLGGATLDNEENYIIKKLFTAAGAVQVENQARI

SEQ ID NO: 44 - DNA, 567 bp, Corynebacterium stationis
  source 1..567: mol_type = genomic DNA
atgtcgaagttaagtccgctgaattggccggttgtgcgccaggtgaagcgcggcgatctgtttggtcgagataaatcaacccagtctgccaaatcggagaacctgcacgggcgcactgtagaggccgacaaagtagttcaatcggtctgcccttactgcgctgtgggctgctcgcagcgggtatatgtcaaagatgaccgcgtcgttcatattgaaggtgactcggactcgcctatttcgcgcggacgtttgtgcccgaaaggcgctgcctctgagcagctggtgaactctgcgacgcgtttgaccaagattaaataccgcgcgcctcatgcaaccgagtggcaagacctagatctcgaaaccgcaatggatatgattgcggaccgttttattgcctcccgccgcaatcagtggcaggactttgatgaaaaaggccgtgttttaaaccgcaccatgggtgtggcaggacttggtggcgccaccttggataatgaggaaaactacattatcaagaagctgtttactgcagctggtgccgtacaagtcgaaaaccaagcacgcatatga

SEQ ID NO: 45 - protein, 470 aa, Corynebacterium stationis
VTISVIDIFSVGVGPSSSHTVGPMRAAKTFMESLPHAPAKVHTELRGSLSATGKGHATDRAVILGLAGWAPLTVPIDAKPLAGSFIPSEGTVEGPAGSVQYSIAFNNKPVPEHPNCLIFSAWDENGEEIATNMEYFSVGGGFVLSRAELDAQLQATHEVPAGMAAAQNNDNAIPYDFSTGDQLLELCDEHDMTIWEIVAANEAVIHREDGGLAKVNAHLDLVWDVMRECVTDGIATKGILPGGLQVNRRAPQLYSQLLEHQDDTASGFSAMEWVNLYALAVNEQNAAGGRVVTAPTNGACGIIPAVLHYARDFLPDFTRETARRFLLTAGAIGMIIKQNASISGAEVGCQGEVGSASSMAAAGLAEILGSSPAQIENAAEIALEHNLGLTCDPVGGLVQIPCIERNAIGAVKSINSARLARMGEGTHYVTLDNAVQTMAETGRDMLTKYKETSIGGLAKTLGLSVSQVEC

SEQ ID NO: 46 - DNA, 1413 bp, Corynebacterium stationis
  source 1..1413: mol_type = genomic DNA
gtgaccattagcgtcattgacatcttttcagtaggcgtggggccttcgtcctcccacaccgttggccccatgcgtgcagcgaaaacctttatggaatctttgccgcatgctcctgccaaagtacatactgagctgcgtggttcactctcagccacgggtaaaggccacgccaccgaccgcgccgtcattttaggccttgccggatgggcgccacttaccgtacctattgacgctaagccgcttgccggcagttttatcccttctgaaggcacagtcgaaggccccgccggcagcgtgcagtattccattgcgttcaacaacaagccggtgcctgagcacccgaactgtttgatatttagcgcctgggatgaaaatggtgaagaaatcgctaccaatatggagtacttctccgtgggcggcggctttgttctctcacgtgcagagctcgatgcgcagctgcaagccacccacgaagttccggcgggtatggcggctgcgcaaaataatgacaacgcaatcccctatgacttcagcaccggtgatcagctcctagagttgtgcgatgagcacgacatgacaatctgggaaatcgtcgctgccaatgaagcagttattcaccgtgaagatggtgggctggccaaggtcaacgcgcacttggatctggtgtgggatgtcatgcgtgagtgtgttactgatggcattgctaccaaggggattttgcccggtggtctgcaggttaatcgtcgtgctccgcaactttatagtcaattgcttgaacaccaagatgatactgcgtcaggcttttctgccatggagtgggtcaacctctatgcactagccgtcaacgagcaaaatgctgccggtggccgcgtggtcactgctccaactaacggtgcctgcggaatcattcccgcggtcttgcactatgcacgagacttcctccccgatttcactcgtgagacagcccggcgttttctgctcaccgctggcgctattggcatgatcatcaagcagaatgcttctatctctggcgctgaggttggctgccaaggagaagtcggctcggcatcgtcaatggctgctgccgggttggctgagattttaggctcgagtccagcacagatcgaaaatgcggcagaaatagcactcgagcacaatctcggtctaacctgcgatccggtcggcggcttggtgcagattccgtgcatcgagcgcaatgcgattggcgcagtaaagtctattaactccgcacgccttgcccgcatgggtgaaggcacgcattacgtcaccctcgataatgctgtgcagacaatggccgagaccggccgagacatgctcaccaagtacaaagagacttcgatcggtggcttggctaagaccctgggactatctgtctcccaggtggagtgctaa

SEQ ID NO: 47 - protein, 952 aa, Corynebacterium stationis
MDFIARHLGPDATESKDMLARVGYDSVEALVTSAIPQSISITDALNMPQALSETDAQAKLRAYADKNVVLKSFYGQGYSDTITPAVIRRGLVEDAGWYTAYTPYQPEISQGRLESLLNFQTMVQDLTGLPIANASLLDEASAVAEAVGLMSRAVKKGRRVLLDARLHPQVLTVAAERARAIDLEVEIADLSNGVVGEDLVGAVVAYTGTEGDIFDPRAVIEEIHGRGGLVSVAADLLSLLLLEGPGSFGADIVIGSSQRFGVPLFFGGPHAAFMAVTDKLKRQMPGRLVGVSVDSEGRPAYRLALQTREQHIRRERATSNICTAQALLANVAAMYAVYHGPEGLKEIANHVHSLAASFAGAVTTQGLKITSSEFFDTVTVAGVDAASIKFSLEKAGYLVRTIGEDKVSVSFGESATQGDVTVLADAFGAAAVDNADFPLPEALTRTTEVLTHEIFNSIHSETQMMRYLRKLGDKDLALDRTMIPLGSCTMKLNPTAAMEPITWPEFANVHPYSPEYATQGWRELIEELEGWLAELTGYAKVSIQPNAGSQGELAGLLAIRRYHVANGDTNRDIVLIPASAHGTNAASATLANLRVVVVKTAEDGSIDLEDLDAKIAKHGQNMAGIMITYPSTHGVFDPEVREVCDKIHAAGGQVYIDGANMNALTGWAQPGKFGGDVSHLNLHKTFTIPHGGGGPGVGPIGVAEHLIPFLPTDAAADELDPANPTPVEQGVPITASQFGSAGVLPITWAYIAMTGGEGLTSATAHAILGANYLARELSDSFPILFTGNEGLVAHECILDLRALTDASGVTAADVAKRLIDFGFHAPTLAFPVAGTLMVEPTESEDIAELDRFIEAMRTIRAEIQEIIDGKIAYEDSVIRHAPYTAPSVSSDDWEYSFSREKAAWPVPSLRLNKYFPPVRRLDEAYGDRNLVCSCPPPEAFDFDADTDSTEEA

SEQ ID NO: 48 - DNA, 2859 bp, Corynebacterium stationis
  source 1..2859: mol_type = genomic DNA
atggatttcattgcccgccaccttgggccagatgccacagaatctaaggacatgctggcgcgtgtgggttatgacagcgtagaagcgcttgtcacctcagcaatcccccagtccattagcatcacggatgcgcttaatatgccgcaggcattgagtgagaccgacgcacaagccaagcttcgcgcttacgctgataaaaatgtcgtgctgaagtctttctacggccagggctactcagacaccatcacccctgctgttattcgccgcggtttggtagaagacgctggttggtacaccgcttataccccataccagccagaaatttcccagggtcgccttgagtcgctgctgaacttccagaccatggttcaagacctcaccggcttgcctattgcgaatgcttctttgctggatgaggcatcggcagttgctgaggccgtgggtttgatgtctcgtgcggtcaagaagggccgccgcgtactgctcgacgcccgtttgcacccacaggttctcaccgtggcggcggagcgtgcccgagcaattgacctcgaagttgagattgctgacttgagcaacggcgtggttggcgaagacctcgtcggcgcagtagttgcctacaccggtacggagggcgatatttttgacccacgtgctgttatcgaagaaatccatggccgcggcggacttgtttccgtcgcggctgacttgttgtccttgctgcttctggaaggcccaggctcgttcggtgcagacattgtcattggttcctcccaacgctttggtgtgccgctcttctttggtggcccacacgctgctttcatggcagtaactgacaagctaaagcgtcagatgccaggccgtttggtcggcgtatcggtcgattctgagggccgtcctgcttaccgcttggcgctgcagactcgtgaacagcacatccgccgtgaacgcgcgacgtcaaatatttgtaccgcgcaggcacttctggccaacgtggctgccatgtacgccgtctaccacggtccagaaggcttgaaggagattgctaaccacgtgcactccttggctgcttcctttgccggtgcagttactactcagggtctgaagattacttcctcggagttcttcgacaccgttaccgttgccggcgttgatgccgcatccattaagttcagcttggaaaaggccggatacctggtgcgcaccattggcgaggataaggtttctgtctccttcggtgagtccgcaacccaaggcgatgttactgtcttggcggacgcctttggtgccgctgcagtagataatgcagatttcccactgcctgaagcactcacccgcaccaccgaggtgctcacccacgaaatctttaactccattcactccgaaacccagatgatgcgttacctgcgcaagctcggtgataaggatctggctctagatcgcaccatgattcctttgggctcatgcaccatgaagctcaacccaaccgcagccatggaaccgatcacctggccagaattcgccaatgttcacccttactcccctgaatacgcaacccagggctggcgtgagctcattgaagagttggaaggctggttggctgagctgaccggctacgccaaggtttctatccaaccaaacgctggttcccagggcgagctagctggtcttttggctatccgccgctaccacgtcgcaaatggtgacaccaaccgcgatatcgtgttgattcctgcgtccgcgcacggcaccaacgctgcctccgcgaccctggcaaatctgcgcgttgttgtggttaagaccgccgaagacggctccatcgatctggaagatctcgatgcgaagatcgccaagcatggtcagaacatggccggaatcatgatcacctacccatccactcacggcgtctttgacccagaggttcgtgaagtctgcgacaagatccatgccgctggcggccaggtctacattgatggcgcaaacatgaatgctttgactggttgggctcagccgggcaagttcggtggcgatgtctcgcacttgaacctgcacaagactttcaccattccgcacggcggtggcggcccaggtgttggaccaattggtgtcgctgagcacctcattccattcctgccaacggatgctgcagctgatgagctggatcctgctaacccaaccccagtagaacagggcgttccaattactgcttcgcagtttggttccgctggtgttctgccgattacctgggcatacatcgcaatgaccggtggcgagggtctaacctccgctactgcacacgccatcttgggtgctaactaccttgcgcgcgaactctccgattccttcccaattctgttcaccggtaatgaaggtcttgttgcgcacgagtgcattttggatctgcgcgcgctaaccgatgcctcaggcgttactgcagcagacgttgccaagcgtttgatcgactttggcttccacgctcctaccctcgcattcccagtggctggcaccttgatggtggaacctactgagtctgaggatattgctgaactggatcgtttcattgaagcaatgcgcaccatccgtgcggagattcaggaaatcatcgatggcaagatcgcatatgaagattcggtcatccgccacgcaccttacaccgcaccgtcagtctcaagcgatgattgggagtactcctttagccgtgaaaaggccgcatggccagttccttcactgcgtttgaacaagtacttcccaccggtacgccgcctggatgaagcttacggcgaccgcaacctggtgtgctcctgcccaccgccagaggcattcgacttcgatgccgacaccgattccaccgaggaggcttaa

SEQ ID NO: 49 - protein, 367 aa, Corynebacterium stationis
MSELRQSPLHAEHEKLGASFTAFGPWNMPLKYGKELDEHHAVRNAVGMFDLSHMGEIWVNGPDAAAFLSYALISNMETVKNGKAKYSMIVAEDGGIIDDLISYRFSDTKFLVVPNAGNTDVVWEAFNQRIEGFDVELNNESLDVAMIALQGPNAAKVLVEQVAEESKEEVENLPYYAATMAKVADVDTIVARTGYTGEDGFELMIYNADATKLWQLFIDQDGVTPCGLASRDSLRLEAGMPLYGNELSRDITPVEAGMGVAFKKKTADFVGAEVLRQRLEEGPKQVIKALTSSERRAARTGAEIYAGEQLVGTVTSGQPSPTLGHPIALALVDTAANLEEGAEVEVDIRGKRYPFTVTKTPFYSREK

SEQ ID NO: 50 - DNA, 1104 bp, Corynebacterium stationis
  source 1..1104: mol_type = genomic DNA
atgtcagaactacgccagtccccactgcacgcagagcacgaaaagctcggcgcatcctttaccgcttttggcccttggaatatgccactaaagtacggcaaggagctcgatgagcaccacgcagtgcgtaatgcagtcggcatgtttgacctctcgcacatgggtgagatttgggtcaacggcccagacgccgctgcatttttgtcctatgcgctgatctccaacatggagaccgtgaaaaatggcaaggcgaagtactccatgattgttgctgaagacggcggcatcatcgatgacctaatttcctaccgtttctccgataccaagttcttggtagtgccaaacgctggcaacactgatgtggtttgggaagcttttaatcagcgcattgaaggcttcgatgtagaactcaacaatgagtccttggatgttgcgatgattgccctgcagggccccaatgctgccaaggttctagttgaacaggttgctgaagagtccaaggaagaagtagaaaaccttccttactatgccgcaaccatggccaaagtcgcagacgttgacaccatcgtcgcgcgcaccggctacaccggcgaagacggcttcgagctgatgatctacaacgccgatgcgaccaagctctggcagcttttcatcgaccaagatggtgttactccatgcggtttagcttcacgcgattccttgcgcttggaagctggcatgcctttgtacggcaatgagctttcccgcgatatcacccctgtcgaggcaggcatgggtgtggcgtttaagaagaagaccgctgacttcgtcggcgccgaggtcctgcgtcaacgcttggaagaaggccctaagcaagttatcaaggctttgacctcctctgagcgccgtgcagcgcgcaccggtgctgaaatctatgccggcgagcagttggtaggcaccgtaacttcgggtcagccatcgccgacgctgggacaccctattgccctggcactggtagatactgcagcaaacctcgaagaaggcgcagaagtagaagtggatattcgcggcaagcgttaccccttcaccgttaccaagacgcctttctatagccgcgagaagtaa

SEQ ID NO: 51 - protein, 129 aa, Corynebacterium stationis
MANLPAEFTYSEDHEWINAAQDAIVGKTVRIGITSVAADRLGEVVFAELPAVGDSVTAGETCGEVESTKSVSDLYSPVTGTVTAVNETVHDDYEIINNDPFGEGWLFEVEVEELGEVMTADEYAAENGI

SEQ ID NO: 52 - DNA, 390 bp, Corynebacterium stationis
  source 1..390: mol_type = genomic DNA
atggctaacctacctgcagaatttacttactccgaagaccacgagtggattaacgccgctcaggacgcaatcgttggcaaaactgttcgcatcggcatcacttctgttgccgcagaccgtcttggtgaggttgtcttcgctgagcttccagcagttggcgatagcgtcactgcaggtgaaacctgtggtgaggttgaatccaccaagtccgtttctgacctgtacagccctgtcaccggtaccgtgaccgctgtgaacgagacagtgcacgatgattatgaaatcatcaacaatgatcctttcggtgaaggttggctgtttgaggtcgaggttgaagaactcggcgaggttatgaccgctgatgaatacgcggcagaaaacggcatctaa

SEQ ID NO: 53 - protein, 433 aa, Corynebacterium stationis
MTTQNSSDAQYQEMRDLDPEVYAAINGEIARQRDTLEMIASENFVPRAVLQAQGSVLTNKYAEGYPGRRYYGGCEHVDIVEDLARDRAKALFGAEFANVQPHSGAQANAAVLASLINPGDKILGLSLAHGGHLTHGMKLNFSGKLYEVAAYEVDAETNRIDMDKLREQAIAEKPQVIIAGWSAYPRTLDFEAYRSIADEVGAYLWTDMAHFAGLVAADLYPNPVPHSDIVSTTVHKTLGGPRSGMILAKQDYAKKLNSAVFPGQQGGPLMHVVAAKAIAMKVAASEEFRDRQVRTLEGAKILAERLTTPEAKAAGVDVLTGGTDVHLVLADLRNSEMDGQQAEDLLHEVGITVNRNAVPNDPRPPMVTSGLRIGTSALATRGLDAEAFTEVADIIGTALTDGKNADTQKLRARVDKLAEQFPLYEGLEDWKIV

SEQ ID NO: 54 - DNA, 1302 bp, Corynebacterium stationis
  source 1..1302: mol_type = genomic DNA
atgactacccagaattcttccgatgctcagtaccaggaaatgcgtgacttagacccagaggtctatgcagcaattaacggtgaaattgctcgtcagcgcgataccctggagatgattgcgtcggagaactttgttcctcgtgcagtcttgcaggcacagggttccgtccttaccaacaagtacgcagagggctacccaggtcgccgctactacggtggatgtgagcacgtcgatatcgtcgaagatctggcgcgtgaccgcgctaaggctctgttcggcgctgagtttgccaatgtacagccacactccggtgcacaggcaaacgctgccgtccttgcttctcttatcaacccaggcgataagatcttgggcctttctttggctcacggtggtcacctgacccacggcatgaagctgaacttctccggcaagctctacgaagtagctgcctacgaagtcgatgcagaaaccaaccgtatcgacatggacaagctgcgtgagcaggctattgcagaaaagccacaggtcatcatcgctggctggtctgcatacccacgcactctggattttgaagcataccgttccatcgcggatgaagtgggggcttacctgtggaccgatatggcacactttgctggtctcgttgccgctgatctgtacccaaatccagttccacactctgacattgtttccaccaccgtgcacaagaccctgggcggtcctcgctccggcatgatcctggctaagcaggactacgctaagaagctcaactctgcagtcttcccaggccagcagggtggccctttgatgcatgtggttgcagcgaaggcaattgccatgaaggttgctgcttccgaagaattccgtgaccgtcaggtccgtactctggaaggcgcgaagattcttgctgagcgcttgaccactcctgaggcaaaggcagcaggcgttgacgttctcactggcggcaccgacgtgcacttggttcttgcggacctgcgcaattctgagatggatggccagcaggcagaagacctcctgcacgaggtcggcatcaccgttaaccgcaacgcggttccaaacgatccacgtccaccaatggtgacctctggtctgcgtatcggtacttccgctctggctacccgcggcctggatgcagaagcattcaccgaggtggcagacatcatcggcaccgcgcttaccgatggcaagaacgccgatacccagaagctgcgcgcacgcgtggacaagcttgctgagcagttcccactctacgagggcttggaagactggaagatcgtctaa

SEQ ID NO: 55 - protein, 422 aa, Corynebacterium stationis
LESYIGSPLTSNAVRVLMLGGGELAKGLVGAFQNLGLEVHVVDRYEGSPAQQVAHFSYTADIDDEKAVLDLVEHIKPAYVVPEIEGVADEALHALHDDSAVTVVPTARACELTSDRKKLREVAESLGLPTTAYKVVETFDALKEAVNELGLPCIIKPDVATSGRGHVLVKDEDQLKDAWDNVRRGKKNSWVVAERFVDFDYEVIIMAVRSIDPETGKLATWFSEPIGYEHARGNLVDCWQPKTMSQRAFENARSVAARISNELGGRGIFAVELFVAGDDIYFSSVTPRPSDKAMLTEATQRFSQYELHARAILGLPIDITLVSPGASSLLHATEEIDEVTYSGVEEALQVAETDVRLFGKPSAYPGRRMGLIMATADDVSEARDRAAIAASKITISAAPRLVPEPELTSEKELSPDEVEISE

SEQ ID NO: 56 - DNA, 1269 bp, Corynebacterium stationis
  source 1..1269: mol_type = genomic DNA
ttggagtcttatatcggtagccccctgacctcgaatgctgttcgggttctcatgctcggcggcggtgagctggccaaaggtttggtgggcgcgtttcagaatttgggcttggaagtccacgttgtcgaccgctatgaggggtctccagcacagcaggttgcacactttagctacaccgcagatatcgatgatgaaaaggccgtgctcgatttagttgagcacatcaagccggcttatgtcgtgccagaaatcgagggcgtagcagatgaggctttgcatgcgcttcacgatgactccgctgtcaccgttgtgcccaccgcccgggcgtgtgagcttaccagcgaccggaagaagctacgcgaagtcgcagaaagcctcggcttgccgacgaccgcgtacaaggtcgtagaaaccttcgacgctttgaaagaagcggtgaacgagctcggtttgccgtgcattattaagccggatgttgcaacctctggacgcgggcatgtgctggtcaaagacgaagaccaactcaaagacgcgtgggataatgtgcgtcgcggcaagaagaactcctgggttgtcgccgaacgctttgtggattttgactatgaagtcatcatcatggcggtgcgctcgattgacccggaaacgggcaagctggcaacgtggttctcagagccgattggttatgagcatgcgcgcggcaacctcgtggactgctggcagccaaagacgatgagccagcgtgcttttgaaaatgcacgttcggttgcagcgcgtatttctaacgaactcggcggccgcggcatcttcgcggtggagctgtttgtcgcgggcgacgatatctacttctcctcggtgaccccgcgtccttctgataaagcgatgctgaccgaagccacccaacgcttttcgcagtatgaattgcacgcgcgcgccattttgggcctgccgatcgacatcacgcttgtctcaccgggcgctagctctttgttgcacgcgaccgaagagatcgacgaagttacctactcgggcgttgaagaagccctgcaggttgcagaaaccgatgtgcgcctattcggcaagccttcggcataccctggccgacgcatggggttgatcatggccaccgccgacgatgtctccgaagcacgcgaccgcgctgcgatcgcggcatcgaagatcacgattagcgccgccccaaggttagttcctgaaccagaactaacctctgaaaaagagttatcccccgatgaggtcgaaatctccgagtaa